European Patent Application EP 4 647 498 A2, published November 12, 2025. Title: IMPROVED REPROGRAMMING METHODS AND CELL CULTURE PLATFORMS. Applicant: FATE THERAPEUTICS, INC. Application WO PCT/US2015/018801, filed March 4, 2015. The sequence listing filed with the application follows.

SEQUENCE LISTING (31 sequences)

SEQ ID NO: 1 - protein, 19 aa, synthetic construct
  REGION 1..19: note = Synthetic made in lab
LLNFDLLKLAGDVESNPGP

SEQ ID NO: 2 - protein, 19 aa, synthetic construct
  REGION 1..19: note = Synthetic made in lab
TLNFDLLKLAGDVESNPGP

SEQ ID NO: 3 - protein, 14 aa, synthetic construct
  REGION 1..14: note = Synthetic made in lab
LLKLAGDVESNPGP

SEQ ID NO: 4 - protein, 17 aa, synthetic construct
  REGION 1..17: note = Synthetic made in lab
NFDLLKLAGDVESNPGP

SEQ ID NO: 5 - protein, 20 aa, synthetic construct
  REGION 1..20: note = Synthetic made in lab
QLLNFDLLKLAGDVESNPGP

SEQ ID NO: 6 - protein, 24 aa, synthetic construct
  REGION 1..24: note = Synthetic made in lab
APVKQTLNFDLLKLAGDVESNPGP

SEQ ID NO: 7 - protein, 40 aa, synthetic construct
  REGION 1..40: note = Synthetic made in lab
VTELLYRMKRAETYCPRPLLAIHPTEARHKQKIVAPVKQT

SEQ ID NO: 8 - protein, 18 aa, synthetic construct
  REGION 1..18: note = Synthetic made in lab
LNFDLLKLAGDVESNPGP

SEQ ID NO: 9 - protein, 40 aa, synthetic construct
  REGION 1..40: note = Synthetic made in lab
LLAIHPTEARHKQKIVAPVKQTLNFDLLKLAGDVESNPGP

SEQ ID NO: 10 - protein, 33 aa, synthetic construct
  REGION 1..33: note = Synthetic made in lab
EARHKQKIVAPVKQTLNFDLLKLAGDVESNPGP

SEQ ID NO: 11 - DNA, 18 bp, synthetic construct
  misc_feature 1..18: note = Primer
  source 1..18: mol_type = other DNA
gcccccaccctttgtgtt

SEQ ID NO: 12 - DNA, 23 bp, synthetic construct
  misc_feature 1..23: note = Primer
  source 1..23: mol_type = other DNA
ttgaaaactttggcttccttgtt

SEQ ID NO: 13 - DNA, 20 bp, synthetic construct
  misc_feature 1..20: note = Primer
  source 1..20: mol_type = other DNA
caggcccgaaagagaaagcg

SEQ ID NO: 14 - DNA, 20 bp, synthetic construct
  misc_feature 1..20: note = Primer
  source 1..20: mol_type = other DNA
ggagggccttggaagcttag

SEQ ID NO: 15 - DNA, 20 bp, synthetic construct
  misc_feature 1..20: note = Primer
  source 1..20: mol_type = other DNA
tatacacaggccgatgtggg

SEQ ID NO: 16 - DNA, 20 bp, synthetic construct
  misc_feature 1..20: note = Primer
  source 1..20: mol_type = other DNA
ttgaccgggaccttgtcttc

SEQ ID NO: 17 - DNA, 20 bp, synthetic construct
  misc_feature 1..20: note = Primer
  source 1..20: mol_type = other DNA
gtggtccgagtgtggttctg

SEQ ID NO: 18 - DNA, 20 bp, synthetic construct
  misc_feature 1..20: note = Primer
  source 1..20: mol_type = other DNA
gttctcctgggccatcttgc

SEQ ID NO: 19 - DNA, 20 bp, synthetic construct
  misc_feature 1..20: note = Primer
  source 1..20: mol_type = other DNA
aagcgcagatcaaaaggaga

SEQ ID NO: 20 - DNA, 20 bp, synthetic construct
  misc_feature 1..20: note = Primer
  source 1..20: mol_type = other DNA
ccccctgaacctgaaacata

SEQ ID NO: 21 - DNA, 19 bp, synthetic construct
  misc_feature 1..19: note = Primer
  source 1..19: mol_type = other DNA
tgcttcccgtatggctttc

SEQ ID NO: 22 - DNA, 22 bp, synthetic construct
  misc_feature 1..22: note = Primer
  source 1..22: mol_type = other DNA
aaagggagatccgactcgtctg

SEQ ID NO: 23 - DNA, 20 bp, synthetic construct
  misc_feature 1..20: note = Primer
  source 1..20: mol_type = other DNA
atcgtcaaagctgcacacag

SEQ ID NO: 24 - DNA, 20 bp, synthetic construct
  misc_feature 1..20: note = Primer
  source 1..20: mol_type = other DNA
cccaggagtcccagtagtca

SEQ ID NO: 25 - DNA, 20 bp, synthetic construct
  misc_feature 1..20: note = Primer
  source 1..20: mol_type = other DNA
gtggacctgacctgccgtct

SEQ ID NO: 26 - DNA, 20 bp, synthetic construct
  misc_feature 1..20: note = Primer
  source 1..20: mol_type = other DNA
ggaggagtgggtgtcgctgt

SEQ ID NO: 27 - DNA, 24 bp, synthetic construct
  misc_feature 1..24: note = Primer
  source 1..24: mol_type = other DNA
gggtttttgggattaagttcttca

SEQ ID NO: 28 - DNA, 22 bp, synthetic construct
  misc_feature 1..22: note = Primer
  source 1..22: mol_type = other DNA
agcctaaatgatggtgcttggt

SEQ ID NO: 29 - skipped

SEQ ID NO: 30 - protein, 7 aa, synthetic construct
  REGION 1..7: note = Polypeptide cleavage recognition site
ENLYFQG

SEQ ID NO: 31 - protein, 7 aa, synthetic construct
  REGION 1..7: note = Polypeptide cleavage recognition site
ENLYFQS